European Patent Application EP 4 389 741 A1, published June 26, 2024. Title: Cyclic peroxides, oxidation reaction products, method for producing oxidation reaction products, and use thereof. Applicant: 株式会社メディプラス製薬. The sequence listing filed with the application follows.

SEQUENCE LISTING (12 sequences)

SEQ ID NO: 1 - DNA, 23 bp, synthetic construct
  misc_feature 1..23: note = profilaggrin_fw primer
  source 1..23: mol_type = other DNA
catggcagctatggtagtgcaga

SEQ ID NO: 2 - DNA, 23 bp, synthetic construct
  misc_feature 1..23: note = profilaggrin_rv primer
  source 1..23: mol_type = other DNA
accaaacgcacttgctttacaga

SEQ ID NO: 3 - DNA, 20 bp, synthetic construct
  misc_feature 1..20: note = involucrin_fw primer
  source 1..20: mol_type = other DNA
gctggagcagcctgtgtttg

SEQ ID NO: 4 - DNA, 20 bp, synthetic construct
  misc_feature 1..20: note = involucrin_rv primer
  source 1..20: mol_type = other DNA
ctggacactgcgggtggtta

SEQ ID NO: 5 - DNA, 22 bp, synthetic construct
  misc_feature 1..22: note = serine palmitoyltransferase_fw primer
  source 1..22: mol_type = other DNA
gcctgtcagcagctcataccaa

SEQ ID NO: 6 - DNA, 23 bp, synthetic construct
  misc_feature 1..23: note = serine palmitoyltransferase_rv primer
  source 1..23: mol_type = other DNA
ggcctgtccagtagaggtaccaa

SEQ ID NO: 7 - DNA, 20 bp, synthetic construct
  misc_feature 1..20: note = GAPDH_fw primer
  source 1..20: mol_type = other DNA
gcaccgtcaaggctgagaac

SEQ ID NO: 8 - DNA, 19 bp, synthetic construct
  misc_feature 1..19: note = GAPDH_rv primer
  source 1..19: mol_type = other DNA
tggtgaagacgccagtgga

SEQ ID NO: 9 - DNA, 20 bp, synthetic construct
  misc_feature 1..20: note = heme oxygenase 1_fw primer
  source 1..20: mol_type = other DNA
ttgccagtgccaccaagttc

SEQ ID NO: 10 - DNA, 20 bp, synthetic construct
  misc_feature 1..20: note = heme oxygenase 1_rv primer
  source 1..20: mol_type = other DNA
tcagcagctcctgcaactcc

SEQ ID NO: 11 - DNA, 22 bp, synthetic construct
  misc_feature 1..22: note = NAD(P)H quinone oxidoreductase 1_fw primer
  source 1..22: mol_type = other DNA
gtggcagtggctccatgtactc

SEQ ID NO: 12 - DNA, 25 bp, synthetic construct
  misc_feature 1..25: note = NAD(P)H quinone oxidoreductase 1_rv primer
  source 1..25: mol_type = other DNA
gagtgtgcccaatgctatatgtcag